European Patent Application EP 4 268 837 A1, published November 1, 2023. Title: Novel modified Reovirus and the uses thereof. Applicant: Virocure Inc. The sequence listing filed with the application follows.

SEQUENCE LISTING (28 sequences)

SEQ ID NO: 1 - protein, 455 aa, Artificial Sequence
  Sigma-1
MDPRLREEVVRLIIALTSDNGVSLSKGLESRVSALEKTSQIHSDTILRITQGLDDANKRIIALEQSRDDLVASVSDAQLAISRLESSIGALQTVVNGLDSSVTQLGARVGQLETGLAELRVDHDNLVARVDTAERNIGSLTTELSTLTLRVTSIQADFESRISTLERTAVTSAGAPLSIRNNRMTMGLNDGLXLSGNNLAIRLPGNTGLNIQNGGLQFRFNTDQFQIVNNNLTLKTTVFDSINSRXGAXEQSXVASAVTPLRLNSSTKVLDMLIDSSTLEINSSGQLTVRSTSPNLRYPIADVSGGIGMSPNYRFRQSMWIGIVSYSGSGLNWRVQVNSDIFIVDDYIHICLPAFDGFSIADGGDLSLNFVTGLLPPLLTGDTEPAFHNDVVTYGAQTVAIGLSSGGAPQYMSKNLWVEQWQDGVLRLRVEGGGSITHSNSKWPAMTVSYPRSFT

SEQ ID NO: 2 - protein, 1289 aa, Artificial Sequence
  Lambda-2
MANVWGVRLADSLSSPTIETRTRQYTLHDLCSDLDANPGREPWKPLRNQRTNNIVAVQLFRPLQGLVLDTQLYGFPGAFDDWERFMREKLRVLKYEVLRIYPISNYSNEHVNVFVANALVGAFLSNQAFYDLLPLLIINDTMIGDLLGTGASLSQFFQSHGDVLEVAAGRKYLQMENYSNDDDDPPLFAKDLSDYAKAFYSDTYEVLDRFFWTHDSSAGVLVHYDKPTNGHHYLLGTLTQMVSAPPYIINATDAMLLESCLEQFSANVRARPAQPVTRLDQCYHLRWGAQYVGEDSLTYRLGVLSLLATNGYQLARPIPRQLTNRWLSSFVSQIMSDGVNETPLWPQERYVQIAYDSPSVVDGATQYGYVRKNQLRLGMRISALQSLSDTPSPVQWLPQYTIDQAAMDEGDLMVSRLTQLPLRPDYGNIWVGDALSYYVDYNRSHRVVLSSELPQLPDTYFDGDEQYGRSLFSLARKIGDRSLVKDTAVLKHAYQAIDPNTGKEYLRSGQSVAYFGASAGHSGADQPLVIEPWIQGKISGVPPPSSVRQFGYDVARGAIVDLARPFPSGDYQFVYSDVDQVVDGHDDLSISSGLVESLLSSCMHATAPGGSFVVKINFPTRPVWHYIEQKILPNITSYMLIKPFVTNNVELFFVAFGVHQHSSLTWTSGVYFFLVDHFYRYETLSTISRQLPSFGYVDDGSSVTGIETISIENPGFSNMTQAARIGISGLCANVGNARKSIAIYESHGARVLTITSRRSPASARRKSRLRYLPLIDPRSLEVQARTILPADPVLFENVSGASPHVCLTMMYNFEVSSAVYDGDVVLDLGTGPEAKILELIPATSPVTCVDIRPTAQPSGCWNVRTTFLELDYLSDGWITGVRGDIVTCMLSLGAAAAGKSMTFDAAFQQLIKVLSKSTANVVLVQVNCPTDVVRSIKGYLEIDSTNKRYRFPKFGRDEPYSDMDALEKICRTAWPNCSITWVPLSYDLRWTRLALLESTTLSSASIRIAELMYKYMPIMRIDIHGLPMEKRGNFIVGQNCSLVIPGFNAQDVFNCYFNSALAFSTEDVNAAMIPQVSAQFDATKGEWTLDMVFSDAGIYTMQALVGSNANPVSLGSFVVDSPDVDITDAWPAQLDFTIAGTDVDITVNPYYRLMTFVRIDGQWQIANPDKFQFFSSASGTLVMNVKLDIADKYLLYYIRDVQSRDVGFYIQHPLQLLNTITLPTNEDLFLSAPDMREWAVKESGNTICILNSQGFVLPQDWDVLTDTISWSPSIPTYIVPPGDYTLTPL

SEQ ID NO: 3 - protein, 708 aa, Artificial Sequence
  Mu-1
MGNASSIVQTINVTGDGNVFKPSAETSSTAVPSLSLSPGMLNPGGVPWIAVGDETSVTSPGALRRMTSKDIPETAIINTDNSSGAVPSESALVPYIDEPLVVVTEHAITNFTKAEMALEXNREFLDKMRVLSVSPKYSDLLTYVDCYVGVSARQALNNFQKQVPVITPTRQTMYVDSIQAALKALEKWEIDLRVAQTLLPTNVPIGEVSCPMQSVVKLLDDQLPDDSLIRRYPKEAAVALAKRNGGIQWMDVSEGTVMNEAVNAVAASALAPSASAPPLEEKSKLTEQAMDLVTAAEPEIIASLXPVPAPVFAIXPKPADYNVRTLRIDEATWLRMIPKSMNTPFQIQVTDNTGTNWHLNLRGGTRVVNLDQIAPMRFXLDLGGKSYKETSWDPNGKKVGFIVFQSKIPFELWTAASQIGQATVVNYVQLYAEDSSFTAQSIIATTSLAYNYEPEQLNKTDPEMNYYLLATFIDSAAITPTNMTQPDVWDALLTMSPLSAGEVTVKGAVVSEVVPADLIGSYTPESLNASLPNDAARCMIDRASKIAEAIKIDDDAGPDEYSPNSVPIQGQLAISQLETGYGVRIFNPKGILSKIASRAMQAFIGDPSTIITQAAPVLSDKNNWIALAQGVKTSLRTKSLSAGVKTAVSKLSSSESIQNWTQGFLDKVSAHFPAPKPDCPTSGDSGESSNRRVKRDSYAGVVKRGYTR

SEQ ID NO: 4 - protein, 365 aa, Artificial Sequence
  Sigma-3
MEVCLPNGHQVVDLINNAFEGRVSIYSAQEGWDKTISAQPDMMVCGGAVVCMHCLGVVGSLQRKLKHLPHHRCNQQIRHQDYVDVQFADRVTAHWKRGMLSFVAQMHEMMNDVSPDDLDRVRTEGGSLVELNXLQVDPNSMFRSIHSSWTDPLQVVDDLDTKLDQYWTALNLMIDSSDLIPNFMMRDPSHAFNGVKLXGDARQTQFSRTFDSRSSLEWGVMVYDYSELEHDPSKGRAYRKELVTPARDFGHFGLSHYSRATTPILGKMPAVFSGMLTGNCKMYPFIKGTAKLKTVRKLVEAVNHAWGVEKIRYALGPGGMTGWYNRTMQQAPIVLTPAALTMFPDTIKFGDLNXPVXIGDPMILG

SEQ ID NO: 5 - protein, 1267 aa, Artificial Sequence
  Lambda-3
MSSMILTQFGPFIESISGITDQSNDVFEDAAKAFSMFTRSDVYKALDEIPFSDDAMLPIPPTIYTKPSHDSYYYIDALNRVRRKTYQGPDDVYVPNCSIVELLEPHETLTSYGRLSEAIENRAKDGDSQARIATTYGRIAESQARQIKAPLEKFVLALLVAEAGGSLYDPVLQKYDEIPDLSHNCPLWCFREICRHISGPLPDRAPYLYLSAGVFWLMSPRMTSAIPPLLSDLVNLAILQQTAGLDPSLVKLGVQICLHAAASSSYAWFILKTKSIFPQNTLHSMYESLEGGYCPNLEWLEPRSDYKFMYMGVMPLSAKYARSAPSNDKKARELGEKYGLSSVVGELRKRTKTYVKHDFASVRYIRDAMACTSGIFLVRTPTETVLQEYTQSPEIKVPIPQKDWTGPIGEIRILKDTTSSIARYLYRTWYLAAARMAAQPRTWDPLFQAIMRSQYVTARGGSGAALRESLYAINVSLPDFKGLPVKAATKIFQAAQLANLPFSHTSVAILADTSMGLRNQVQRRPRSIMPLNVPQQQVSAPHTLTADYINYHMNLSTTSGSAVIEKVIPLGVYASSPPNQSINIDISACDASITWDFFLSVIMAAIHEGVASSSIGKPFMGVPASIVNDESVVGVRAARPISGMQNMIQHLSKLYKRGFSYRVNDSFSPGNDFTHMTTTFPSGSTATSTEHTANNSTMMETFLTVWGPEHTDDPDVLRLMKSLTIQRNYVCQGDDGLMIIDGTTAGKVNSETIQKMLELISKYGEEFGWKYDIAYDGTAEYLKLYFIFGCRIPNLSRHPIVGKERANSSAEEPWPAILDQIMGVFFNGVHDGLQWQRWIRYSWALCCAFSRQRTMIGESVGYLQYPMWSFVYWGLPLVKAFGSDPWIFSWYMPTGDLGMYSWISLIRPLMTRWMVANGYVTDRCSPVFGNADYRRCFNELKLYQGYYMAQLPRNPKKSGRAAPREVREQFTQALSDYLMQNPELKSRVLRGRSEWEKYGAGIIHNPPSLFDVPHKWYQGAQEAAIATREELAEMDETLMRARRHSYSSFSKLLEAYLLVKWRMCEAREPSVDLRLPLCAGIDPLNSDPFLKMVSVGPMLQSTRKYFAQTLFMAKTVSGLDVNAIDSALLRLRTLGADKKALTAQLLMVGLQESEADALAGKIMLQDVNTVQLARVVNLAVPDTWMSLDFDSMFKHHVKLLPKDGRHLNTDIPPRMGWLRAILRFLGAGMVMTATGVAVDIYLEDIHGGGRSLGQRFMTWMRQEGRSA

SEQ ID NO: 6 - protein, 1275 aa, Artificial Sequence
  Lambda-1
MKRIPRKTKGKSSGKGNDSTERADDGSSQLRDKQNNKAGPATTEPGTSNREQYKARPGIASVQRATESAEMPMKNNDEGTPDKKGNTKGDLVNEHSEAKDEADEATKKQAKDTDKSKAQVTYSDTGINNANELSRSGNVDNEGGSNQKPMSTRIAEATSAIVSKHPARVGLPPTASSGHGYQCHVCSAVLFSPLDLDAHVASHGLHGNMTLTSSDIQRHITEFISSWQNHPIVQVSADVENKKTAQLLHADTPRLVTWDAGLCTSFKIVPIVPAQVPQDVLAYTFFTSSYAIQSPFPEAAVSRIVVHTRWASNVDFDRDSSVIMAPPTENNIHLFKQLLNTETLSVRGANPLMFRANVLHMLLEFVLDNLYLNRHTGFSQDHTPFTEGANLRSLPGPDAEKWYSIMYPTRMGTPNVSKICNFVASCVRNRVGRFDRAQMMNGAMSEWVDVFETSDALTVSIRGRWMARLARMNINPTEIEWALTECAQGYVTVTSPYAPSVNRLMPYRISNAERQISQIIRIMNIGNNATVIQPVLQDISVLLQRISPLQIDPTIISNTMSTVSESTTQTLSPASSILGKLRPSNSDFSSFRVALAGWLYNGVVTTVIDDSSYPKDGGSVTSLENLWDFFILALALPLTTDPCAPVKAFMTLANMMVGFETIPMDNQIYTQSRRASAFSTPHTWPRCFMNIQLISPIDAPILRQWAEIIHRYWPNPSQIRYGAPNVFGSANLFTPPEVLLLPIDHQPANVTTPTLDFTNELTNWRARVCELMKNLVDNQRYQPGWTQSLVSSMRGTLDKLKLIKSMTPMYLQQLAPVELAVIAPMLPFPPFQVPYVRLDRDRVPTMVGVTRQSRDTITQPALSLSTTNTTVGVPLALDARAITVALLSGKYPPDLVTNVWYADAIYPMYADTEVFSNLQRDMITCEAVQTLVTLVAQISETQYPVDRYLDWIPSLRASAATAATFAEWVNTSMKTAFDLSDMLLEPLLSGDPRMTQLAIQYQQYNGRTFNIIPEMPGSVIADCVQLTAEVFNHEYNLFGIARGDIIIGRVQSTHLWSPLAPPPDLVFDRDTPGVHIFGRDCRISFGMNGAAPMIRDETGLMVPFEGNWIFPLALWQMNTRYFNQQFDAWIKTGELRIRIEMGAYPYMLHYYDPRQYANAWNLTSAWLEEITPTSIPSVPFMVPISSDHDISSAPAVQYIISTEYNDRSLFCTNSSSPQTIAGPDKHIPVERYNILTNPDAPPTQIQLPEVVDLYNVVTRYAYETPPITAVVMGVP

SEQ ID NO: 7 - protein, 721 aa, Artificial Sequence
  MuNS
MASFKGFSANTVPVSKAKRDISSLAATPGLRSQSFTPSVDMSQSREFLTKAIEQGSMSIPYQHVNVPKVDRKVVSLVVRPFSSGAFSISGVISPAHAYLLECLPQLEQAMAFVASPESFQASDVAKRFAIKPGMSLQDAITAFINFVSAMLKMTVTRQNFDVIVAEIERLASTSVSVRTEEAKVADEELMLFGLDHRGPQQLDVSDAKGIMKAADIQTTHDVHLAPGVGNIDPEIYNEGRFMFMQHKPLAADQSYFTLETADYFKIYPTYDEHDGRMADQKQSGLILCTKDEVLAEQTIFKLDAPDDKTVHLLDRDDDHVVARFTKVFIEDVAPGHHAAQRSGQRSVLDDLYANTQVISITSAALKWVVKHGVSDGIVNRKNVKVCVGFDPLYTLSTHNGVSLCALLMDEKLSVLNSACRMTLRSLMKTGRDVDAHRAFQRVLSQGYTSLMCYYHPSRKLAYGEVLFLERSNDVTDGIKLQLDASRQCHECPVLQQKVVELEKQIIMQKSIQSDPTPVALQPLLSQLRELSSEVTRLQMELSRAQSLNAQLEADVKSAQSCSLDMYLRHHTCINGHAKEDELLDAVRVAPDVRREIMEKRSEVRQGWCERISKEAAAKCQTVIDDLTLMNGKQAQEITELRDSAEKYEKQIAELVSTITQNQITYQQELQALVAKNVELDALNQRQAKSLRITPSLLSATPXDSXXGVADLIDFSVPTDEL

SEQ ID NO: 8 - protein, 418 aa, Artificial Sequence
  Sigma-2
MARAAFLFKTVGFGGLQNVPINDELSSHLLRAGNSPWQLTQFLDWISLGRGLATSALVPTAGSRYYQMSCLLSGTLQIPFRPNHRWGDIRFLRLVWSAPTLDGLVVAPPQVLAQPALQAQADRVYDCDDYPFLARDPRFKHRVYQQLSAVTLLNLTGFGPISYVRVDEDMWSGDVNQLLMNYFGHTFAEIAYTLCQASANRPWEYDGTYARMTQIVLSLFWLSYVGVIHQQNTYRTFYFQCNRRGDAAEVWILSCSLNHSAQIRPGNRSLFVMPTSPDWNMDVNLILSSTLTGCLCSGSQLPLIDNNSVPAVSRNIHGWTGRAGNQLHGFQVRRMVTEFCDRLRRDGVMTQAQQNQVEALADQTQQFKRDKLETWAREDDQYNQAHPNSTMFRTKPFTNAQWGRGNTGATSAAIAALI

SEQ ID NO: 9 - DNA, 1416 bp, Artificial Sequence
  S1 segment
gctattggtcggatggatcctcgcctacgtgaagaagtagtacggctgataatcgcattaacgagtgataatggagtatcactgtcaaaagggcttgaatcaagggtctcggcgctcgagaagacgtctcaaatacactctgatactatcctccggatcacccagggactcgatgatgcaaacaaacgaatcatcgctcttgagcaaagtcgggatgacttggttgcatcagtcagtgatgctcaacttgcaatctccagattggaaagctctatcggagccctccaaacagttgtcaatggacttgattcgagtgttacccagttgggtgctcgagtgggacaacttgagacaggacttgcagagctacgcgttgatcacgacaatctcgttgcgagagtggatactgcagaacgtaacattggatcattgaccactgagctatcaactctgacgttacgagtaacatccatacaagcggatttcgaatctaggatatccacattagagcgcacggcggtcactagcgcgggagctcccctctcaatccgtaataaccgtatgaccatgggattaaatgatggactcaygttgtcagggaataatctcgccatccgattgccaggaaatacgggtctgaatattcaaaatggtggacttcagtttcgatttaatactgatcaattccagatagttaataataacttgactctcaagacgactgtgtttgattctatcaactcaaggabaggcgcaaytgagcaaagtkmcgtggcgtcggcagtgactcccttgagattaaacagtagcacgaaggtgctggatatgctaatagacagttcaacacttgaaattaattctagtggacagctaactgttagatcgacatccccgaatttgaggtatccgatagctgatgttagcggcggtatcggaatgagtccaaattataggtttaggcagagcatgtggataggaattgtctcctattctggtagtgggctgaattggagggtacaggtgaactccgacatttttattgtagatgattacatacatatatgtcttccagcttttgacggtttctctatagctgacggtggagatctatcgttgaactttgttaccggattgttaccaccgttacttacaggagacactgagcccgcttttcataatgacgtggtcacatatggagcacagactgtagctatagggttgtcgtcgggtggtgcgcctcagtatatgagtaagaatctgtgggtggagcagtggcaggatggagtacttcggttacgtgttgaggggggtggctcaattacgcactcaaacagtaagtggcctgccatgaccgtttcgtacccgcgtagtttcacgtgaggatcagaccaccccgcggcactggggcatttcatc

SEQ ID NO: 10 - DNA, 3916 bp, Artificial Sequence
  L2 segment
gctaaaaggcgcgatggcgaacgtttggggggtgagacttgcagactcgttatcttcacccactattgagacacgaacgcgtcagtataccttacacgatctttgctcagacctagatgctaatccggggagggaaccgtggaaacctctgcgtaatcagcgtactaataatattgtggctgtgcaattattcagaccattgcagggtttagttttagatacccagctttatggatttccaggagcatttgatgactgggagcgattcatgagagagaagctgcgtgtgctaaagtatgaagtattgcgcatctatccaatcagcaactatagcaatgaacatgtcaacgtcttcgtggccaatgctttggtgggcgctttcctgtcgaatcaagctttctatgacctgctaccgttgttgataattaatgacactatgattggtgatctacttggcacgggggcatcgctatcacagttctttcaatctcatggagatgtgctggaagtcgcagctggtcgtaagtatctgcagatggaaaactactccaacgatgacgatgatcctccattatttgcgaaagacctgtcagattatgctaaagcattctacagtgacacatatgaagtgttggacaggttcttttggacgcatgactcttcagcgggggtcttagtgcattatgataagccaacgaatggtcatcactatctgctgggtactttgactcagatggtcagtgcacctccttatattattaacgctactgacgcaatgttgcttgaatcctgtctagaacagttctcagctaatgtgcgtgcgagacctgcgcaacccgttacacgcttagaccaatgctatcatttaagatggggagcacaatatgtaggagaagattcactgacatatcggttgggggtgttatccttgctggctaccaatggatatcaattagctagaccgattccaagacagttgacgaatcgatggttgtcgagctttgtgagtcaaattatgtctgacggcgtcaacgagactccactgtggccccaagaaaggtatgtgcagatcgcttatgattcaccatccgttgttgatggggctacgcaatatggctatgtcaggaagaatcaactcagactcggcatgagaatatcggcgctgcaatcgctgagtgatacgccctcgccggtacagtggcttccacaatacaccatcgaccaggcagcgatggacgaaggcgatctgatggttagtcggcttacgcaactcccgttacgtcctgattatggtaatatctgggtcggcgatgcgctatcctattatgtggactacaatcggagtcatcgagtcgtgctttcatcggaacttcctcagcttccggacacatattttgatggcgatgaacagtatgggcgcagcctgttctcactagctcgtaagattggtgaccgctcgttagtgaaagatacggctgtcttgaagcacgcttaccaagccatcgatccaaatactggtaaggagtatctgagatctgggcaatctgtcgcatattttggtgcatcagcgggtcattctggtgccgaccagccgttagtcatagagccctggattcaagggaaaatcagtggtgtgccgccaccctcctcagtgcgacagttcggctatgatgttgcccgtggcgcgatcgtcgatctggcgagaccatttccttctggagattatcaatttgtctattcggatgttgaccaggtggtcgatggccatgacgatctgagtatatcatctggactggtggagagccttttgtcttcatgcatgcacgccacagcacccgggggctcatttgttgttaagataaattttccgactagacccgtatggcactacatcgaacagaagatcttgcccaatattacgtcatacatgttgatcaagcctttcgtcaccaacaacgtcgaattgttcttcgtcgctttcggtgtgcatcaacactcatcacttacttggacatctggagtgtacttcttcttggtggaccatttttatcgttatgagactttatctacgatctcacgacaattgccgtcttttgggtatgttgatgatgggtcttccgtgactggtatcgagacaattagtattgagaaccctggcttctcgaatatgacccaggccgctcgcattggtatctcaggattgtgtgctaatgtaggtaacgcgcgtaagtccattgccatttacgaatcccatggggccagagtattaactatcacatcaaggagatctccggcatcagctagaagaaagtctaggttgcgatatttgccattaatagaccctaggtcgttagaggtacaggcgcgcactattctgccagctgatccagtgttatttgaaaacgtgagcggagcgtcaccccatgtttgtctgacaatgatgtacaacttcgaagtgtcgtcagcggtatatgatggagacgttgtgctagatcttgggacgggaccagaggctaaaatccttgaactgatacccgcaacctctccagtcacatgcgtggacatacggcctacagcgcagcctagtggatgttggaacgttcgtaccacgttccttgagttagattatttgagcgatggatggatcactggggtgcgtggggacatagttacttgtatgttatctttgggggccgctgccgctggaaaatcaatgacttttgacgctgcgtttcagcaattaatcaaagtattatccaagagtacggctaatgttgtgctggtgcaggttaactgccctacagacgtggtgaggagcattaagggctacctagagatagattcgactaacaagaggtataggttccccaaatttggtcgagacgagccgtactctgacatggatgcgctggagaaaatatgtcgtaccgcctggccaaactgctcaattacctgggttccattgtcatacgacttgcggtggactagactggcattattagagtccacgacattgagtagcgcgtcgattagaattgctgagctgatgtataaatacatgcctattatgaggattgatattcatggactacccatggaaaagcgaggtaacttcatagtggggcagaactgctcattagtaatccctggttttaatgcgcaggatgtctttaactgttatttcaattccgccctcgctttctcgactgaagatgtcaatgctgcgatgattccccaagtgtctgcgcagtttgatgcgactaagggtgagtggacgttggatatggtcttctccgacgcaggaatctataccatgcaggctctagtgggatctaatgctaatccagtctctttgggttcctttgtagttgattctccagatgtagatataactgacgcttggccagctcagttagactttacgatcgcgggaactgatgtcgatataacagttaatccttattaccgtctgatgacctttgtaaggatcgatggacagtggcagattgccaatccagacaaatttcaattcttttcgtcggcgtctgggacgttagtgatgaacgtcaaattagatatcgcagataaatatctactatactatatacgagatgtccagtctcgagatgttggcttttacattcagcatccacttcaacttttgaatacgatcacattgccaaccaacgaggacctttttctgagcgcacctgacatgcgagagtgggcagttaaggaaagcggtaacacgatatgtatactcaatagtcaagggtttgtgctacctcaagattgggatgtgttaacagataccataagttggtccccatcgatacccacatacattgtgccaccgggtgattataccttgactcctctgtaactcactgtccctcgtgagcgcgcctaattcatc

SEQ ID NO: 11 - DNA, 2203 bp, Artificial Sequence
  M2 segment
gctaatctgctgaccgttactctgcaaagatggggaacgcttcctctatcgttcagacgatcaacgtcactggagatggcaatgtatttaaaccatcagctgaaacttcatctaccgctgtaccatcgttaagcttatcacctggaatgctgaatcccggaggggtaccatggattgctgttggagatgagacatctgtgacttcaccaggcgcattacgtcgaatgacgtcaaaggacatcccggaaacggcaataatcaacacagacaattcatcaggcgccgtgccaagcgaatcagccttggtgccctacatcgatgagccgctggtagtggttacagagcatgctattaccaacttcaccaaagctgagatggcacttgaawtcaatcgtgagttccttgacaagatgcgtgtgctgtcagtgtcaccaaaatattcggatcttctgacctatgttgactgctacgtcggtgtgtctgctcgtcaggctttaaacaattttcagaaacaagtgcctgtgattacacctactaggcagacgatgtatgtcgactcgatacaagcggccttgaaagctttagaaaagtgggagattgatctgagagtggctcaaacgttgctgcctacgaacgttccgattggagaagtctcttgtccaatgcagtcggtagtgaaactgctggatgatcagctgccagatgacagcctgatacggaggtatcccaaggaagccgccgtcgctttggctaaacgaaacgggggaatacaatggatggacgtatcagaaggcaccgtgatgaacgaggctgtcaacgctgttgcagctagtgcactggcaccttcagcatcagccccacccttagaagagaagtcaaagttaaccgaacaagcgatggatctcgtgaccgcggctgagcctgagataattgcctcactcgygccagttcccgcacccgtgtttgccataycacctaaaccagcagattataatgtgcgtactctgaggatcgacgaggccacttggctgcgaatgattccaaaatcaatgaacacaccttttcaaatccaggtgactgataacacaggaactaattggcatctcaatttgaggggggggactcgtgtagtgaatctggaccaaatcgctccgatgcggtttgyattagatctagggggaaagagttataaagagacgagctgggatccaaacggcaagaaggtcggattcatcgtttttcaatcgaagataccattcgaactttggactgctgcttcacagatcggtcaagccacggtggttaactatgtccaactatacgctgaagacagctcatttaccgcgcagtctatcattgctactacctctttggcttataactatgagcctgagcagttgaataagactgaccctgagatgaattattatcttttggcgacctttatagactcagccgctataacgccaacgaatatgacacagcctgatgtttgggatgccttgctgacgatgtccccactatcagctggcgaggtgacagtgaagggtgcggtagtgagtgaagtagtccctgcagacttgataggtagctacactccagaatccctaaacgcctcacttccgaatgatgctgctagatgcatgatcgatagagcttcgaagatagccgaagcaatcaagattgatgatgatgctggaccagatgaatattccccaaactctgtaccaattcaaggtcagcttgctatctcgcaactcgaaactggatatggtgtgcgaatattcaaccctaaagggatcctttctaaaattgcatctagggcaatgcaggctttcattggtgacccgagcacaatcatcacgcaggcggcgccagtgttatcagacaagaataattggattgcattggcacagggagtgaaaactagtctgcgtactaaaagtctatcagcgggagtgaagactgcagtgagtaagctgagctcatctgagtctatccagaattggactcaaggattcttggataaagtgtcagcgcattttccagcaccaaagcccgattgtccgactagcggagatagtggtgaatcgtctaatcgccgagtgaagcgcgactcatacgcaggagtggtcaaacgtgggtacacacgttaggccgctcgccctggtgacgcggggttaagggatgcaggcaaatcatc

SEQ ID NO: 12 - DNA, 1196 bp, Artificial Sequence
  S4 segment
gctatttttgcctcttcccagacgttgtcgcaatggaggtgtgcttgcccaacggtcatcaggtcgtggacttgattaacaacgcttttgaaggtcgtgtatcaatctacagcgcgcaagagggatgggacaaaacaatctcagcacagccagatatgatggtatgtggtggcgccgtcgtttgcatgcattgtctaggtgttgttggatctctacaacgcaagctgaagcatttgcctcaccatagatgtaatcaacagatccgtcatcaggattacgtcgatgtacagttcgcagaccgtgttactgctcactggaagcggggtatgctgtccttcgttgcgcagatgcacgagatgatgaatgacgtgtcgccagatgacctggatcgtgtgcgtactgagggaggttcactagtggagctgaacyggcttcaggttgacccaaattcaatgtttagatcaatacactcaagttggacagatcctttgcaggtggtggacgaccttgacactaagctggatcagtactggacagccttaaacctgatgatcgactcatccgacttgatacccaactttatgatgagagacccatcacacgcgttcaatggtgtgaaactggrgggagatgctcgtcaaacccaattctccaggacttttgattcgagatcgagtttggaatggggtgtgatggtttatgattactctgagctggagcatgatccatcgaagggccgtgcttacagaaaggaattggtgacgccagctcgagatttcggtcactttggattatcccattattctagggcgactaccccaatccttggaaagatgccggccgtattctcaggaatgttgactgggaactgtaaaatgtatccattcattaaaggaacggctaagctgaagacagtgcgcaagctagtggaggcagtcaatcatgcttggggtgtcgagaagattagatatgctcttgggccaggtggcatgacgggatggtacaataggactatgcaacaggcccccattgtgctaactcctgctgctctcacaatgttcccagataccatcaagtttggggatttgaattrtccagtgaygattggcgatccgatgattcttggctaaacacccccatcttcacagcgccgggcttgaccaacctggtgtgacgtgggacaggcttcattcatc

SEQ ID NO: 13 - DNA, 3860 bp, Artificial Sequence
  L1 segment
gctacacgttccacttccacgacaatgtcatccatgatactgactcagtttggaccgttcattgagagcatttcaggtatcactgatcaatcgaatgacgtgtttgaagatgcagcaaaagcattctctatgtttactcgcagcgatgtctacaaggcgctggatgaaatacctttctctgatgatgcgatgcttccaatccctccaactatatatacgaaaccatctcacgattcatattattacattgatgctctaaaccgtgtgcgtcgcaaaacatatcagggccctgatgacgtgtacgtacctaattgttctattgttgaattgctggagccacatgagactctgacatcttatgggcggttgtccgaggccatcgagaatcgtgccaaggatggggacagccaagccagaatcgccacaacgtatggtagaatcgctgaatctcaagctcgacagattaaggctccattggagaagtttgtgttggcactattagtggccgaagcaggggggtctttatatgatccagttttgcagaagtatgatgagattccagatctatcgcataattgccctttatggtgttttagagagatctgtcgtcacatatctggtccattaccagatcgggcaccttatctttacttatctgcaggggttttctggttaatgtcaccacgaatgacgtctgcaatccctccgctactatccgatcttgttaatttagctattttgcaacaaactgcgggtttagatccatcattagtgaaattgggagtacagatatgccttcatgcagcagctagctcaagttatgcatggtttatcttaaagactaagtctatttttcctcaaaacacgttgcacagtatgtatgaatctctagaagggggatactgtcctaatcttgaatggttagagcctagatcagactataagttcatgtacatgggagtcatgccattgtccgctaagtatgctaggtcggcgccgtccaatgataagaaagcgcgggaacttggcgagaaatatggactgagctcagtcgtcggtgagcttcgtaaacggacaaagacgtatgttaaacatgactttgcttcagtgaggtacattcgtgacgctatggcatgtactagcggtattttcttggtaagaacacccaccgaaacggtattgcaagaatatacgcagagtccggagattaaggttcccattccccagaaagactggacaggcccaataggtgaaatcagaattctaaaagatacaacaagttccatcgcgcgttacttatatagaacatggtacttggcagcggcgagaatggcggctcaaccacgtacgtgggatccattgtttcaagcgattatgagatctcaatacgtgacagctaggggtggatctggcgcagcactccgcgaatctttgtatgcaatcaatgtgtcgttacctgatttcaagggcttaccagtgaaggcagcaactaagatattccaggcggcacaattagcgaacttgccgttctcccacacatcagtggctatactagctgacacttcaatgggattgcgaaatcaggtgcagaggcggccacgatccattatgccattaaatgtgccccagcagcaggtttcggcgccccatacattgacagcggattacattaactaccacatgaatctatcaaccacgtctggtagtgcggtcattgagaaggtgattcctttaggtgtatacgcttcgagccctcctaaccagtcgatcaacattgacatatctgcgtgtgacgctagtattacttgggatttctttctgtcagtgattatggcggctatacacgaaggtgtcgctagtagctccattggaaaaccatttatgggggttcctgcatccattgtaaatgatgagtctgtcgttggagtgagagctgctaggccgatatcgggaatgcagaacatgattcagcatctatcgaaactatataaacgtggattttcatatagagtaaacgattctttttctccaggtaacgattttactcatatgactaccactttcccgtcaggttcaacagccacctctactgagcatactgctaataatagtacgatgatggaaactttcctgacagtatggggacccgaacatactgacgaccctgacgtcttacgtttaatgaagtctttaactattcaaaggaattacgtatgtcaaggtgatgatggattaatgattatcgatgggactactgctggtaaggtgaacagtgaaactattcagaagatgctagaattaatctcaaaatatggtgaggaattcggatggaaatatgacatagcgtacgatgggactgccgaatacttaaagctatacttcatatttggctgtcgaattccaaatcttagtcgccatccaatcgtggggaaagaacgggcgaattcttcagcagaggagccatggccagcaattctagatcagattatgggtgtcttctttaatggtgttcatgatgggttacagtggcagcggtggatacgttattcatgggctctatgctgtgctttctcacgtcaaagaacaatgattggtgagagcgtgggttaccttcaatatcctatgtggtcttttgtctactggggattaccactggttaaagcgtttgggtcagacccatggatattttcttggtacatgcctactggagatctgggaatgtatagttggattagcttgatacgccctctgatgacaagatggatggtggctaatggttacgtaactgacagatgctcacccgtattcgggaacgcagattatcgcaggtgtttcaatgaacttaaactatatcaaggttattatatggcacaattgcccaggaatcctaagaagtctggacgagcggcccctcgggaggtaagagaacaattcactcaggcattatccgactatctaatgcaaaatccagagctgaagtcacgtgtgctacgtggtcgtagtgagtgggagaaatatggagcggggataattcacaatcctccgtcattattcgatgtgccccataaatggtatcagggtgcgcaagaggcagcaatcgctacgagagaagagctggcagaaatggatgagacattaatgcgcgctcgaaggcacagctattcgagcttttcaaagttattagaggcgtatctgctcgtgaaatggcgaatgtgcgaggcccgcgaaccgtcggttgatttgcgattaccattatgtgcgggtattgacccattaaactcagatccttttctcaagatggtaagcgttggaccaatgctccagagtacgagaaagtactttgctcagacactattcatggcaaagacggtgtcgggtcttgacgttaacgcgattgatagcgcgttattacgactgcgaacattaggtgctgataagaaagcattaacggcgcagttattaatggtggggcttcaggagtcagaagcggacgcattggccgggaagataatgctacaggatgtgaatactgtgcaattagccagagtggttaacttagctgtgccagatacttggatgtcgttagactttgaytctatgttcaaacaccacgtcaagctgcttcccaaagatggacgtcatctaaatactgatattcctcctcgaatgggatggttacgggccattttacgattcttaggtgccggaatggtaatgactgcgactggagttgctgtcgacatctatctggaggatatacatggcggtggtcggtcacttggacagagattcatgacttggatgcgacaggaaggacggtcagcgtgagtctaccatgggtcgtggtgcgtcaactcatc

SEQ ID NO: 14 - DNA, 3901 bp, Artificial Sequence
  L3 segment
gctaatcgtcaggatgaagcggattccaaggaagacaaagggcaaatccagcggaaagggcaatgactcaacagagagagcggacgatggctcgagccaattaagagacaagcaaaacaataaggctggccccgccactacggagcctggcacatccaaccgagagcaatacaaagctcgaccaggtattgcatctgtgcagagggccactgaaagtgcagaaatgcccatgaagaataatgacgaagggacgccagataagaaaggaaatactaagggcgacctagttaatgagcatagtgaggctaaagacgaggcggatgaagcgacgaagaagcaggcaaaggatacagacaaaagtaaagcgcaagtcacatattcagacactggtatcaataatgctaatgaactgtcaagatctgggaatgtggataatgagggtggaagtaatcagaagccgatgtctaccagaatagctgaggcaacgtctgctatagtgtcgaaacatcctgcgcgtgttgggctgccacctaccgctagcagtggtcatgggtatcagtgccatgtctgttctgcagtcctgtttagtcctttagacctagatgcccacgtcgcctcacatggtttgcatggtaacatgacattaacatcgagtgatatccagcgacatataactgagttcatcagctcatggcaaaatcatcctattgttcaagtttcggctgatgtcgaaaataagaaaactgctcaattgcttcacgctgacactcctcgactcgtcacttgggatgctggtttgtgtacttcattcaaaatcgtcccgattgtgccagctcaggtgccgcaggatgtactggcctatacgtttttcacctcttcatacgctatccaatcaccgtttccagaggcggcagtgtctaggattgtggtgcatacgagatgggcatctaatgttgactttgaccgagactcgtctgtcatcatggcgccacctacagaaaacaatatccatttgtttaaacagttactaaatactgaaaccctgtctgtaaggggggctaatccgctaatgttcagggcgaatgtgttgcatatgttgctagagttcgtattagataacttgtatctgaacagacatacgggattctctcaagaccacacgccatttactgagggtgctaatttgcgttcacttcctggccccgatgctgagaaatggtactcgattatgtatccaacgcgcatgggaacgccgaatgtatccaaaatatgtaatttcgtcgcctcttgtgtgcgaaatcgggttggacggtttgatcgagcacagatgatgaacggagctatgtcagagtgggtggatgtcttcgagacttcagacgcgctaaccgtctccattcgaggtcgatggatggctagactagctcgcatgaacataaatccaacagagatcgaatgggcattgactgaatgtgcacaaggatatgtgactgtcacaagtccttacgctcctagcgtaaatagattgatgccctatcgtatctccaacgctgagcggcaaatatcacagataatcaggatcatgaacattggcaataacgcgacggtgatacaacctgttctgcaagatatttcggtactccttcaacgcatatcaccactccaaatagatccaactattatttccaacactatgtcaacagtctcggagtctactactcagaccctcagccccgcgtcctcaattttgggtaaactacgaccaagcaactcagatttttctagttttagagtcgcgttggctggatggctttataatggggttgtgacgacggtgattgatgatagttcatatccaaaagacggcggcagcgtgacctcacttgaaaatctgtgggatttcttcatccttgcgcttgctctaccactgacaactgacccctgtgcacctgtgaaagcattcatgaccctagccaacatgatggttggtttcgagacaatccctatggataatcagatctatactcaatcgagacgcgcgagtgctttctcaacgcctcacacgtggccacgatgctttatgaacatccagttaatttctccaatcgacgctcccatcttgcgacagtgggctgaaattattcatagatactggcctaacccttcacagattcgttatggtgcaccgaacgttttcggctcggcaaatttgttcactccacctgaggtgctgttattgccaatcgatcatcaaccagctaatgtaacaacgccaacgctggacttcaccaatgagttaactaattggcgcgctcgtgtctgtgagcttatgaagaatctcgttgataaccaaagatatcaacctggatggacacaaagtctagtctcgtcaatgcgcggaacgctagacaaattgaagttgattaaatcgatgacaccaatgtatctgcaacagctggctccggtagagttagcagtgatagctcccatgttgccttttccacctttccaggtgccatacgtccgtctcgatcgtgacagagttccaacaatggttggagtaacacgacagtcacgagatactattactcagccggcgctatcgctgtcgacaaccaatactactgttggcgtgccactagctctagacgcgagggctatcaccgttgcgctgttgtcagggaaatatccgccggatttggtgacaaatgtatggtacgctgatgccatttacccaatgtatgcagacacggaggtgttctctaatcttcagagagacatgattacctgcgaggccgtgcagacattagtgactctggtggcgcaaatatcagagacccagtatcctgtagataggtatcttgattggatcccatcactgagagcatcggcggcgacggcggcgacatttgctgagtgggttaatacttcaatgaagacggcgtttgatttgtctgatatgctgttagagcctctcctaagcggtgatccgaggatgactcaactagcgattcagtatcagcagtacaatggcagaacgtttaatatcatacctgaaatgccaggttcagtaattgctgactgcgttcaattaacagcagaagtctttaatcacgaatataacctgtttgggattgcgcggggtgatatcatcattggccgtgttcagtcgacacatttgtggtcaccgctggctcctccacctgacctggtgtttgatcgtgatacccctggtgttcacatcttcggacgagattgccgtatatcgtttggaatgaatggcgccgcgccaatgattagagatgagactggactgatggtgccttttgaaggaaattggattttcccactggcgctttggcaaatgaatacacgatattttaatcaacagttcgacgcgtggattaagacaggagagttgcgaatccgcattgagatgggcgcgtatccatatatgttgcattactatgatccacgtcagtacgctaatgcatggaatttaacatccgcctggcttgaagaaattacgccgacgagcatcccatccgtgcctttcatggtgcccatttcaagtgatcatgacatttcctctgccccagctgtccaatatatcatttcaactgaatataatgatcggtctctgttctgcactaactcatcatctccccaaaccatcgctggaccagacaaacacattccagttgagagatataacattctgaccaaccccgacgctccacccacgcagatacaactgcctgaagtcgttgacttgtacaacgtcgtcacacgctatgcgtatgagactccgcctattaccgctgttgttatgggtgttccttgatcctcatcctcccaacaggtgctagagcattgcgctcaatgctagttgggccgattcatc

SEQ ID NO: 15 - DNA, 2241 bp, Artificial Sequence
  M3 segment
gctaaagtgaccgtggtcatggcttcattcaagggattctccgccaacactgttccagtttctaaggccaagcgtgacatatcatctcttgccgctactcctggacttcgttcacaatccttcactccgtctgtggatatgtctcaatcgcgtgaattcctcacaaaggcaattgagcaagggtccatgtctataccttatcagcatgtgaatgtaccgaaagttgatcgtaaagttgttagcctggtagtgcgacctttctcttcaggtgctttctctatctctggagtgatttcgccagcccatgcctatctactagagtgtctaccccagcttgagcaggcgatggcttttgttgcttcacctgagtctttccaggcttccgacgtcgcgaagcgctttgccataaagccaggtatgagcctccaggatgccatcactgcctttattaactttgtgtccgcgatgctgaaaatgacggtgactcgtcaaaactttgacgttattgtggctgagatcgagaggcttgcttcaaccagcgtgtccgtcaggactgaagaagcgaaggttgctgatgaggagctaatgctattcgggttagatcatagagggccacagcagctggatgtttctgacgctaaagggataatgaaggctgctgatattcagacaactcatgatgtccatttggcaccaggcgttggtaatattgatcctgaaatctataacgaggggcggttcatgttcatgcagcacaagccacttgcggcggatcaatcgtatttcaccttggagactgcggattatttcaagatttatccaacatacgatgaacatgatggcaggatggctgaccaaaagcagtcgggattgatactgtgtactaaggacgaggtattggctgagcaaactatatttaaactggacgcccctgatgacaagactgttcatctgttggatcgcgatgacgaccacgttgttgccagatttactaaggtatttatagaggacgtggctcccgggcatcatgctgctcaaagatcgggacaacgctctgtgcttgatgacctatatgcgaatacgcaagtgatttccattacttctgctgctttaaagtgggtggtcaagcacggcgtatctgatggaatcgtgaacaggaagaatgtcaaagtgtgtgttggttttgaccccctgtacaccttgtctacacataacggggtgtccttatgtgccctgctgatggacgaaaaactctctgtgctgaacagtgcgtgtcgtatgacgttacgctcactcatgaagaccggacgcgacgttgatgcacacagagcttttcagcgagtcctctctcaaggatacacatcgctaatgtgctactatcatccttcacggaagttggcatatggtgaggtgctctttctagaacgatccaatgacgtgacagatgggatcaagcttcagttggacgcatctagacagtgtcatgaatgtcctgtgttgcagcagaaagtggttgagttagagaaacagattattatgcagaagtcaatccagtcagaccctaccccagtggcgctgcaaccattgttgtctcagttgcgtgagttgtctagtgaagttactaggctacagatggagttgagtcgagctcagtccctgaatgctcagttggaggcggatgtcaagtcagctcaatcatgtagcttggatatgtatctgagacaccacacttgcattaatggtcatgctaaagaagatgaattgcttgacgctgtgcgtgtcgcgccggatgtgaggagagaaatcatggaaaagaggagtgaagtgagacaaggttggtgcgaacgtatttctaaggaagcagctgccaaatgtcaaactgttattgatgacctgactttgatgaatggaaagcaagcacaagagataacagaattacgtgattcggctgaaaaatatgagaaacagattgcagagctggtgagtaccatcacccaaaaccagataacgtatcagcaagagctacaagccttggtagcgaaaaatgtggaattggacgcgttgaatcagcgtcaggctaagtctttgcgtattactccctctcttctatcagccactcctabcgattcagytgmtggtgttgctgacttaattgatttctctgttccaactgatgagttgtaaataatccgtgatgcagtgttgccctaatcccttaagccttcccgacccccattcatc

SEQ ID NO: 16 - DNA, 1331 bp, Artificial Sequence
  S2 segment
gctattcgctggtcagttatggctcgcgctgcgttcctattcaagactgttgggtttggtggtctgcaaaatgtgccaattaacgacgaactatcttcacatctactccgagctggtaattcaccatggcagttaacacagtttttagactggataagccttgggaggggtttagctacatcggctctcgttccgacggctgggtcaagatactatcaaatgagttgccttctaagtggcactctccagattccgttccgtcctaaccaccgatggggagacattaggttcttacgcttagtgtggtcagctcctactctcgatggattagtcgtagctccaccacaagttttggctcagcccgctttgcaagcacaggcagatcgagtgtacgactgcgatgattatccatttctagcgcgtgatccaagattcaaacatcgggtgtatcagcaattgagtgctgtaactctacttaacttgacaggttttggcccgatttcctacgttcgagtggatgaagatatgtggagtggagatgtgaaccagcttctcatgaactatttcgggcacacgtttgcagagattgcatacacattgtgtcaagcctcggctaataggccttgggaatatgacggtacatatgctaggatgactcagattgtgttatccttgttctggctatcgtatgtcggtgtaattcatcagcagaatacgtatcggacattctattttcagtgtaatcggcgaggtgacgccgctgaggtgtggattctttcttgttcgttgaaccattccgcacaaattagaccgggtaatcgtagcttattcgttatgccaactagcccagattggaacatggacgtcaatttgatcctgagttcaacgttgacggggtgtttgtgttcgggttcacagctgccactgattgacaataattcagtacctgcagtgtcgcgtaacatccatggctggactggtagagctggtaaccaattgcatgggttccaggtgagacgaatggtgactgaattttgtgacaggttgagacgcgatggtgtcatgacccaagctcagcagaatcaagttgaagcgttggcagatcagactcaacagtttaagagggacaagctcgaaacgtgggcgagagaagacgatcaatataatcaggctcatcccaactccacaatgttccgtacgaaaccatttacgaatgcgcaatggggacgaggtaatacgggggcgactagtgccgcgattgcagcccttatctgatcgtcttggagtgagggggtccccccacacccctcacgactgaccacacattcatc

SEQ ID NO: 17 - DNA, 25 bp, Artificial Sequence
  S1 Primer FW
atggatcctcgcctacgtkaagaag

SEQ ID NO: 18 - DNA, 23 bp, Artificial Sequence
  S1 Primer RV
ctgatcctcacgtgaaactacgc

SEQ ID NO: 19 - DNA, 3860 bp, Artificial Sequence; identical to SEQ ID NO: 13
  Wild-type Reovirus_L1

SEQ ID NO: 20 - DNA, 3916 bp, Artificial Sequence; identical to SEQ ID NO: 10
  Wild-type Reovirus_L2

SEQ ID NO: 21 - DNA, 3901 bp, Artificial Sequence; identical to SEQ ID NO: 14
  Wild-type Reovirus_L3

SEQ ID NO: 22 - DNA, 2224 bp, Artificial Sequence
  Wild-type Reovirus_M1
cgtttggagtagacgctggggctgacgcgaatgacgtttcatatcaagatcatgactatgtgttggatcagttacagtacatgttagatggatatgaggctggtgacgttatcgatgcactcgtccacaagaattggttacatcactctgtctattgcttgttgccacccaaaagtcaactattagagtattggaaaagtaatccttcagcgataccggacaacgttgatcgtcggcttcgtaaacgactaatgctaaagaaagatctcaggaaagatgatgaatacaatcagctagcgcgtgctttcaagatatcggatgtctacgcacctctcatctcatccacgacgtcaccgatgacaatgatacagaacttgaatcaaggcgagatcgtgtacaccacgacggacagggtaataggggctagaatcttgttatatgctcctagaaagtactatgcgtcaactctgtcatttactatgactaagtgcatcattccgtttggtaaagaggtgggtcgtgttcctcactctcgatttaatgttggcacatttccgtcaattgctaccccgaaatgttttgtcatgagtggggttgatattgagtccatcccaaatgaatttatcaagttgttttaccagcgcgtcaagagtgttcacgctaacatactaaatgacatatctcctcagatcgtctctgacatgataaacagaaagcgtctgcgcgttcatactccatcagatcgtcgagccgcgcagttgatgcatttgccttaccatgttaaacgaggagcgtctcacgtcgacgtttacaaggtggatgttgtagacatgttgttcgaggtagtggatgtggccgatgggttgcgcaacgtatctaggaaactaactatgcataccgttccggtatgtattcttgaaatgttgggtattgagattgcggactattgcattcgtcaagaggatggaatgctcacagattggttcctacttttaaccatgctatctgatggcttgactgatagaaggacgcattgtcaatacttgattaatccgtcaagtgtgcctcctgatgtgatacttaacatctcaattactggatttataaatagacatacaatcgatgtcatgcctgacatatatgacttcgttaaacccattggcgctgtgctgcctaagggatcatttaaatcaacaattatgagagttcttgattcaatatcaatattaggaatccaaatcatgccgcgcgcgcatgtagttgactcagatgaggtgggcgagcaaatggagcctacgtttgagcaggcggttatggagatatacaaagggattgctggcgttgactcgctggatgatctcatcaagtgggtgctgaactcggatctcattccgcatgatgacaggcttggtcaattatttcaagcgtttttgcctctcgcaaaggacttattagctccaatggccagaaagttttatgataactcaatgagtgagggtagattgctaacattcgctcatgccgacagtgagttgctgaacgcaaattattttggtcatttattgcgactaaaaataccatatattacagaggttaatctgatgattcgcaagaatcgtgagggtggagagctatttcagcttgtgttatcttatctatataaaatgtatgctactagcgcgcagcctaaatggtttggatcattattgcgattgttaatatgtccctggttacatatggagaaattaataggagaagcagacccggcatctacgtcggctgaaattgggtggcatatccctcgtgaacagctgatgcaagatggatggtgtggatgtgaagacggattcattccctatgttagcatacgtgcgccaagactggttatagaggagttgatggagaagaactggggccaatatcatgcccaagttattgtcactgatcagcttgtcgtaggcgaaccgcggagggtatctgctaaggctgtgatcaagggtaaccacttaccagttaagttagtttcacgatttgcatgtttcacattgacggcgaagtatgagatgaggctttcgtgcggccatagcactggacgtggagctgcatacagtgcgagactagctttccgatctgacttggcgtgatccgtgacatgcgtagtgtgacacctgctcctaggtcaatgggggtagggggcgggctaagactacgtacgcgcttcatc

SEQ ID NO: 23 - DNA, 2203 bp, Artificial Sequence; identical to SEQ ID NO: 11
  Wild-type Reovirus_M2

SEQ ID NO: 24 - DNA, 2241 bp, Artificial Sequence; identical to SEQ ID NO: 15
  Wild-type Reovirus_M3

SEQ ID NO: 25 - DNA, 1416 bp, Artificial Sequence; identical to SEQ ID NO: 9
  Wild-type Reovirus_S1

SEQ ID NO: 26 - DNA, 1331 bp, Artificial Sequence; identical to SEQ ID NO: 16
  Wild-type Reovirus_S2

SEQ ID NO: 27 - DNA, 1198 bp, Artificial Sequence
  Wild-type Reovirus_S3
gctaaagtcacgcctgtcgtcgtcactatggcttcctcactcagagctgcgatctccaagatcaagagggatgacgtcggtcagcaagtttgtcctaattatgtcatgctgcggtcctctgtcacaacaaaggtggtacgaaatgtggttgagtatcaaattcgtacgggcggattcttttcgtgcttagctatgctaaggccactccagtacgctaagcgtgagcgtttgcttggtcagaggaatctggaacgtatatcgactagggatatccttcagactcgtgatttacactcactatgtatgccaactcctgatgcgccaatgtctaatcatcaagcatccaccatgagagagctgatttgcagttacttcaaggtcgatcatgcggatgggttgaaatatatacccatggatgagagatactctccgtcatcacttgccagattgtttaccatgggcatggctgggctgcacattaccactgagccatcttataagcgtgttccgattatgcacttagctgcggacttggactgtatgacgctggctctaccttacatgattacgcttgatggtgatactgtggttcctgtcgctccaacactgtcagcggaacagcttctggacgacggactcaaaggattagcatgcatggatatctcctatggatgtgaggtggacgcgaatagccggccggctggtgatcagagtatggactcttcacgctgcatcaacgagttgtattgcgaggagacagcagaagccatctgtgtgcttaagacatgccttgtgttaaattgcatgcagtttaaacttgagatggatgacctagcacataacgctgctgagctggacaagatacagatgatgatacccttcagtgagcgtgtttttaggatggcctcgtcctttgcgactattgatgcccagtgttttaggttttgcgtgatgatgaaggataaaaatctgaaaatagatatgcgtgaaacgacgagactgtggactcgttcagcatcagatgattctgtggccacgtcatctttaagtatttccctggaccggggtcgatgggtggcggctgacgccagtgatgctagactgctggtttttccgattcgcgtgtaatgggtgagtgagctgatgtggtcgccaagacatgtgccggtgtcttggtggtgggtgacgcctaatcatc

SEQ ID NO: 28 - DNA, 1196 bp, Artificial Sequence; identical to SEQ ID NO: 12
  Wild-type Reovirus_S4